European Patent Application EP 4 353 739 A1, published April 17, 2024. Title: 一种多肽、融合型多聚体蛋白质及其用途. Applicant: 西安蓝晓科技新材料股份有限公司. The sequence listing filed with the application follows.

SEQUENCE LISTING (7 sequences)

SEQ ID NO: 1 - protein, 58 aa, synthetic construct
ADNKFNKEQQNAFYEILHLPNLTEEQRNGFIQSLKDDPSVSKEILAEAKKLNDAQAPK

SEQ ID NO: 2 - protein, 58 aa, synthetic construct [sequence omitted]

SEQ ID NO: 3 - protein, 15 aa, synthetic construct
GGHLIAGGSDSERKE

SEQ ID NO: 4 - protein, 73 aa, synthetic construct
VDNKFNKEQQNAFYEILHLPGGHLIAGGSDSERKENLNEEQRNAFIQSLKDDPSQSANLLAEAKKLNDAQAPK

SEQ ID NO: 5 - protein, 14 aa, synthetic construct
SGDGDGDGSITSKG

SEQ ID NO: 6 - protein, 392 aa, synthetic construct
ADNKFNKEQQNAFYELLHLPNLTEKQRNAFIQSLKDDPSVSKEILAEARKLNDAQAPGADNKFNKEQQNAFYELLHLPNLTEKQRNAFIQSLKDDPSVSKEILAEARKLNDAQAPGADNKFNKEQQNAFYELLHLPNLTEKQRNAFIQSLKDDPSVSKEILAEARKLNDAQAPGADNKFNKEQQNAFYELLHLPNLTEKQRNAFIQSLKDDPSVSKEILAEARKLNDAQAPGSGDGDGDGSITSKGVDNKFNKEQQNAFYEILHLPGGHLIAGGSDSERKENLNEEQRNAFIQSLKDDPSQSANLLAEAKKLNDAQAPKVDNKFNKEQQNAFYEILHLPGGHLIAGGSDSERKENLNEEQRNAFIQSLKDDPSQSANLLAEAKKLNDAQAPK

SEQ ID NO: 7 - DNA, 1176 bp, synthetic construct
  source 1..1176: mol_type = other DNA
gcggataataaatttaacaaggaacagcagaacgcgttttacgagctcttacacctgccgaatctcaccgaaaaacagcgcaacgctttcatccagtctctgaaagatgatccctcggttagtaaagaaattctggcagaagcacgcaaacttaatgacgcacaggcccctaaggccgataacaaatttaacaaggaacagcagaacgcgttttacgaactgctgcacctgccgaacctgactgaaaagcagcgcaatgcattcattcaaagccttaaagatgatccgagcgtttcgaaagagatacttgcggaagctcgcaaactcaacgacgcccaagcgccgaaggctgacaacaaattcaataaagagcagcaaaatgccttctatgagctgttacacctcccgaacctgaccgaaaaacagcgcaatgccttcatccagtcactgaaagacgatccgagcgtctccaaagaaattctagccgaagcgcgtaaactgaacgatgcgcaagcccctaaagccgataataaattcaacaaagagcagcagaatgccttctatgaactgttgcatctcccgaacttaacagaaaaacaacgtaatgcctttatccagtcattgaaggatgacccaagtgtatccaaagaaattcttgcagaagcccggaaactgaacgacgcccaggcaccaggcagcggtgatggtgatggagacggctcgattacgtctaaaggcgtggacaataaatttaacaaagagcagcagaacgcgttttatgaaattttacatctaccgggcggtcatttaatcgcgggcggatccgactcggagcgtaaagaaaatttgaatgaagagcagcgaaacgcatttattcaaagcctgaaggatgatccgagccagtcagcgaacctgctggcggaagcaaagaaattaaatgatgcccaggcgccaaaagtggataataaattcaacaaagagcaacaaaacgcgttttacgaaatcttgcacttgcccgggggccatttaattgcgggtgggagcgactctgaaaggaaggaaaatcttaatgaggaacaacgtaacgcttttattcagagtctgaaggatgatccgagccaatcagcgaatctgctggcagaagcgaaaaaactgaatgatgctcaggcgcctaag